European Patent Specification EP 3 473 706 B1, published September 10, 2025. Title: CELL-EMBEDDED  BEADS FOR HAIR REGROWTH AND THERE USEOF. Applicant: Yokohama National University. The sequence listing filed with the application follows.

SEQUENCE LISTING (10 sequences)

SEQ ID NO: 1 - DNA, 17 bp, Artificial Sequence
  Forward primer for Versican
gacgactgtcttggtgg

SEQ ID NO: 2 - DNA, 17 bp, Artificial Sequence
  Reverse primer for Versican
atatccaaacaagcctg

SEQ ID NO: 3 - DNA, 20 bp, Artificial Sequence
  Forward primer for GAPDH
agaacatcatccctgcatcc

SEQ ID NO: 4 - DNA, 20 bp, Artificial Sequence
  Reverse primer for GAPDH
tccaccaccctgttgctgta

SEQ ID NO: 5 - DNA, 20 bp, Artificial Sequence
  Forward primer for Igfbp5
atgagacaggaatccgaaca

SEQ ID NO: 6 - DNA, 20 bp, Artificial Sequence
  Reverse primer for Igfbp5
tcaacgttactgctgtcgaa

SEQ ID NO: 7 - DNA, 20 bp, Artificial Sequence
  Forward primer for Tgfb2
tcccgaataaaagcgaagag

SEQ ID NO: 8 - DNA, 20 bp, Artificial Sequence
  Reverse primer for Tgfb2
aagcttcgggatttatggtg

SEQ ID NO: 9 - DNA, 22 bp, Artificial Sequence
  Forward primer for HIF1a
ggagatccttcgaggagcactt

SEQ ID NO: 10 - DNA, 25 bp, Artificial Sequence
  Reverse primer for HIF1a
ggcgatttagcagcagatataagaa